European Patent Specification EP 3 260 142 B1, published April 26, 2023. Title: A cartilage regeneration material and a method for production thereof. Applicant: FUJIFILM Corporation. The sequence listing filed with the application follows.

SEQUENCE LISTING (10 sequences)

SEQ ID NO: 1 - protein, 571 aa, Recombinant
GAPGAPGLQGAPGLQGMPGERGAAGLPGPKGERGDAGPKGADGAPGAPGLQGMPGERGAAGLPGPKGERGDAGPKGADGAPGKDGVRGLAGPIGPPGERGAAGLPGPKGERGDAGPKGADGAPGKDGVRGLAGPIGPPGPAGAPGAPGLQGMPGERGAAGLPGPKGERGDAGPKGADGAPGKDGVRGLAGPPGAPGLQGAPGLQGMPGERGAAGLPGPKGERGDAGPKGADGAPGAPGLQGMPGERGAAGLPGPKGERGDAGPKGADGAPGKDGVRGLAGPIGPPGERGAAGLPGPKGERGDAGPKGADGAPGKDGVRGLAGPIGPPGPAGAPGAPGLQGMPGERGAAGLPGPKGERGDAGPKGADGAPGKDGVRGLAGPPGAPGLQGAPGLQGMPGERGAAGLPGPKGERGDAGPKGADGAPGAPGLQGMPGERGAAGLPGPKGERGDAGPKGADGAPGKDGVRGLAGPIGPPGERGAAGLPGPKGERGDAGPKGADGAPGKDGVRGLAGPIGPPGPAGAPGAPGLQGMPGERGAAGLPGPKGERGDAGPKGADGAPGKDGVRGLAGPPG

SEQ ID NO: 2 - protein, 4 aa, Artificial Sequence
  Description of Artificial Sequence: adhesive sequence
REDV

SEQ ID NO: 3 - protein, 5 aa, Artificial Sequence
  Description of Artificial Sequence: adhesive sequence
YIGSR

SEQ ID NO: 4 - protein, 5 aa, Artificial Sequence
  Description of Artificial Sequence: adhesive sequence
PDSGR

SEQ ID NO: 5 - protein, 7 aa, Artificial Sequence
  Description of Artificial Sequence: adhesive sequence
RYVVLPR

SEQ ID NO: 6 - protein, 6 aa, Artificial Sequence
  Description of Artificial Sequence: adhesive sequence
LGTIPG

SEQ ID NO: 7 - protein, 10 aa, Artificial Sequence
  Description of Artificial Sequence: adhesive sequence
RNIAEIIKDI

SEQ ID NO: 8 - protein, 5 aa, Artificial Sequence
  Description of Artificial Sequence: adhesive sequence
IKVAV

SEQ ID NO: 9 - protein, 4 aa, Artificial Sequence
  Description of Artificial Sequence: adhesive sequence
DGEA

SEQ ID NO: 10 - protein, 4 aa, Artificial Sequence
  Description of Artificial Sequence: adhesive sequence
ERGD